European Patent Specification EP 3 613 438 B1, published January 21, 2026. Title: CONJUGATE OF ISOTRETINOIN AND PEPTIDE. Applicant: CAREGEN CO., LTD. The sequence listing filed with the application follows.

SEQUENCE LISTING (31 sequences)

SEQ ID NO: 1 - protein, 14 aa, Artificial Sequence
  Peptide 1
RRLIDRTNANFLVM

SEQ ID NO: 2 - DNA, 20 bp, Artificial Sequence
  forward primer for cEBP-alpha
tcggtggacaagaacagcaa

SEQ ID NO: 3 - DNA, 20 bp, Artificial Sequence
  reverse primer for cEBP-alpha
ccttgaccaaggagctctca

SEQ ID NO: 4 - DNA, 20 bp, Artificial Sequence
  forward primer for PPAR-gamma
ttcgctgatgcactgcctat

SEQ ID NO: 5 - DNA, 20 bp, Artificial Sequence
  reverse primer for PPAR-gamma
acagactcggcactcaatgg

SEQ ID NO: 6 - DNA, 20 bp, Artificial Sequence
  forward primer for SREBP1c
gaccgacatcgaaggtgaag

SEQ ID NO: 7 - DNA, 21 bp, Artificial Sequence
  reverse primer for SREBP1c
aagagaggagctcaatgtggc

SEQ ID NO: 8 - DNA, 20 bp, Artificial Sequence
  forward primer for GAPDH
ggagccaaaagggtcatcat

SEQ ID NO: 9 - DNA, 20 bp, Artificial Sequence
  reverse primer for GAPDH
gtgatggcatggactgtggt

SEQ ID NO: 10 - DNA, 21 bp, Artificial Sequence
  forward primer for ACC
gaatgtttggggatatttcag

SEQ ID NO: 11 - DNA, 21 bp, Artificial Sequence
  reverse primer for ACC
ttctgctatcagtctgtccag

SEQ ID NO: 12 - DNA, 20 bp, Artificial Sequence
  forward primer for aP2
catcagcgtaaatggggatt

SEQ ID NO: 13 - DNA, 20 bp, Artificial Sequence
  reverse primer for aP2
acacattccaccaccagctt

SEQ ID NO: 14 - DNA, 20 bp, Artificial Sequence
  forward primer for IFN-gamma
gaggtcaacaacccacaggt

SEQ ID NO: 15 - DNA, 20 bp, Artificial Sequence
  reverse primer for IFN-gamma
gggacaatctcttccccacc

SEQ ID NO: 16 - DNA, 20 bp, Artificial Sequence
  forward primer for IL-1beta
ttcgacacatgggataacga

SEQ ID NO: 17 - DNA, 20 bp, Artificial Sequence
  reverse primer for IL-1beta
tctttcaacacgcaggacag

SEQ ID NO: 18 - DNA, 20 bp, Artificial Sequence
  forward primer for IL-6
aaagaggcactgccagaaaa

SEQ ID NO: 19 - DNA, 20 bp, Artificial Sequence
  reverse primer for IL-6
atctgaggtgcccatgctac

SEQ ID NO: 20 - DNA, 24 bp, Artificial Sequence
  forward primer for IL-17A
ggtcaacctcaaagtctttaactc

SEQ ID NO: 21 - DNA, 24 bp, Artificial Sequence
  reverse primer for IL-17A
ttaaaaatgcaagtaagtttgctg

SEQ ID NO: 22 - DNA, 21 bp, Artificial Sequence
  forward primer for TNF-alpha
aacatccaaccttcccaaacg

SEQ ID NO: 23 - DNA, 21 bp, Artificial Sequence
  reverse primer for TNF-alpha
gaccctaagcccccaattctc

SEQ ID NO: 24 - DNA, 20 bp, Artificial Sequence
  forward primer for CPT1a
cgtaccaagtagccaaggca

SEQ ID NO: 25 - DNA, 20 bp, Artificial Sequence
  reverse primer for CPT1a
caggaacgcacagtctcagt

SEQ ID NO: 26 - DNA, 19 bp, Artificial Sequence
  forward primer for Acox
ccgccgagagatcgagaac

SEQ ID NO: 27 - DNA, 20 bp, Artificial Sequence
  reverse primer for Acox
cagttgcctggtgaagcaag

SEQ ID NO: 28 - DNA, 17 bp, Artificial Sequence
  forward primer for HSL
ggacacacacacacctg

SEQ ID NO: 29 - DNA, 20 bp, Artificial Sequence
  reverse primer for HSL
ccctttcgcagcaactttag

SEQ ID NO: 30 - DNA, 20 bp, Artificial Sequence
  forward primer for ATGL
tcgtggatgttggtggagct

SEQ ID NO: 31 - DNA, 19 bp, Artificial Sequence
  reverse primer for ATGL
tgtggcctcattcctccta